European Patent Specification EP 2 585 478 B1, published September 20, 2023. Title: A Plant. Applicant: The University of Warwick. The sequence listing filed with the application follows.

SEQUENCE LISTING (62 sequences)

SEQ ID NO: 1 - DNA, 1372 bp, Brassica rapa
atggcgacagaggatgtgaacgaagcccttgcggcggcggaagtaccggcaacagagacgacggagaagcagcctgctcacaagctcgaaagaaagtggagtttctggttcgataaccaatccaaaccaaagcaaggcgccgcctggggagcctcccttcgcaaagcctataccttcgacaccgtccaagacttctgggggtttgtttgtcttctccttttatttattgttagcgatctgtaaagctagatcttcttttgcagtttgcacgagactatattcatccctagcaaactgacgccgaatgctgaaattcacatgttcaaagctggtgttgagcctaagtgggaagatcctgagtgtgctaatgggggaaagtggacttatgttgtcacctccaaccgcaagcctgctttagacaaggcttggcttgaaactgtactcctcttctacctctcctccttttttctttttttttgcatctggtaatgacatgttttctctgccagttgatggctcttgtcggagagcaatttgatgaggctgatgagatttgtggcgtggttgctagtgtgcgcccaaagcaggacaagctctccttgtggacaaggaccaaatctaatgaagctgttctggtatgatgcttgtcttctctcactatgtacctttggtgttgtttgataactgttttcttctacttgttatccgttgcgatgtcccattattgtttgattatcctgttccaatttttttgtattgcgtactggtggtttacgaagaagtgttcttgtacaatatgttagcgttgttgaatgtgttaattgcttactatagtaaaacagtttaagctgttgactatgttaatattctcttcgatacacacacttagaatggataactaccttgtttctttatcctttggagtttcaccagcttattatcgatcgagatactccttctgatttgaattaccattcaagattaatatttatatatattgaaagtatatgtttgtttaacgatatatctattaggcttgctttttttagttcattcgcagtataaacgtagctctatttattagaggcttctctttagaacttggcagtaatgtaatatgtcgaagtgtggtttatgaatctggttgatgatattactaatttttttgtttgttattgtaaatccagatgggtattgggaagaagtggaaggagatacttgatgtcaccgacaagataactttcactaaccatgtaacttaactttctccacatagaggctaattatcttttgttcttcttacgtggcttactaaaatgtggtctacttatatatataggatgattctagaagaactaggttcactgtctga

SEQ ID NO: 2 - RNA, 600 nt, Brassica rapa
auggcgacagaggaugugaacgaagcccuugcggcggcggaaguaccggcaacagagacgacggagaagcagccugcucacaagcucgaaagaaaguggaguuucugguucgauaaccaauccaaaccaaagcaaggcgccgccuggggagccucccuucgcaaagccuauaccuucgacaccguccaagacuucugggguuugcacgagacuauauucaucccuagcaaacugacgccgaaugcugaaauucacauguucaaagcugguguugagccuaagugggaagauccugagugugcuaaugggggaaaguggacuuauguugucaccuccaaccgcaagccugcuuuagacaaggcuuggcuugaaacuuugauggcucuugucggagagcaauuugaugaggcugaugagauuuguggcgugguugcuagugugcgcccaaagcaggacaagcucuccuuguggacaaggaccaaaucuaaugaagcuguucugauggguauugggaagaaguggaaggagauacuugaugucaccgacaagauaacuuucacuaaccaugaugauucuagaagaacuagguucacugucuga

SEQ ID NO: 3 - protein, 199 aa, Brassica rapa
MATEDVNEALAAAEVPATETTEKQPAHKLERKWSFWFDNQSKPKQGAAWGASLRKAYTFDTVQDFWGLHETIFIPSKLTPNAEIHMFKAGVEPKWEDPECANGGKWTYVVTSNRKPALDKAWLETLMALVGEQFDEADEICGVVASVRPKQDKLSLWTRTKSNEAVLMGIGKKWKEILDVTDKITFTNHDDSRRTRFTV

SEQ ID NO: 4 - DNA, 1321 bp, Brassica rapa
atggcgacagaggatgtgaacgaagcccttgcggcggcggaagtaccggcaacagagacgacggagaagcagcctgctgacaagctcgaaagaaagtggagtttctggttcgataaccaatccaaaccaaagcaaggcgccgcctggggagcctcccttcgcaaagcctataccttcgacaccgtccaagacttctggggggtttgtttgtcttctccttttacttattgttagcgatctgtaaagctagatcttcttttgcagtttgcacgagactatattcatccctagcaaactgacgccgaatgctgaaattcacatgttcaaagctggtgttgagcctaagtgggaagatcctgagtgtgctaatggcggaaagtggacttttgttgttacctccaaccgcaagcctgctttagacaaggcttggcttgaaactgtactcatcttctacctctcctctttttttttttaatagtttagacaattttgcatctggtaatgacatgttttatctgccagttgatggctcttgtcggagagcaatttgatgaggctgatgagatctgtggggtggttgctagtgtgcgcccaaagcaggacaagctctccttgtggacaaggaccaaatctaatgaagctgttctggtatgatgcttctcttctctcactatgtacctttggtgttgttttcttctacttgttatccgttgcgatgtcccattattgtttgattatcctgttccaatttttctgttttgcgtactggtggtttacgaagaagtatgcttgtacaatatgttagcgttgttgaatgtgttaattgcttactatagtaaaacagtttaagctgttgactatgttaatattctcttcgatacacacacttagaatggataactaccttgtttctttatcctttggagtttcaccagcttaatatatattgaaagtatatgtttgttcaacgatatatctattaggcttgctttttttagttcattcgcagtataaacatagctctatttattagaggccatctctttagaacttggcagtactgtaatatgtcgaagtgtggtttatgaatctggctgatgatattactactttgttgtttgttattgtaaatccagatgggtattgggaagaagtggaaggagatacttgatgtcaccgacaagataactttcactaaccatgtaacttaactttctccacatagaggctaattatcttttgttcttcttacgtggcttactaaaatgtggtctacttatatatataggatgattctagaagaactcggttcactgtctga

SEQ ID NO: 5 - RNA, 664 nt, Brassica rapa
auggcgacagaggaugugaacgaagcccuugcggcggcggaaguaccggcaacagagacgacggagaagcagccugcugacaagcucgaaagaaaguggaguuucugguucgauaaccaauccaaaccaaagcaaggcgccgccuggggagccucccuucgcaaagccuauaccuucgacaccguccaagacuucugggggguuuguuugucuucuccuuuuacuuauuguuagcgaucuguaaagcuagaucuucuuuugcaguuugcacgagacuauauucaucccuagcaaacugacgccgaaugcugaaauucacauguucaaagcugguguugagccuaagugggaagauccugagugugcuaauggcggaaaguggacuuuuguuguuaccuccaaccgcaagccugcuuuagacaaggcuuggcuugaaacuuugauggcucuugucggagagcaauuugaugaggcugaugagaucuguggggugguugcuagugugcgcccaaagcaggacaagcucuccuuguggacaaggaccaaaucuaaugaagcuguucugauggguauugggaagaaguggaaggagauacuugaugucaccgacaagauaacuuucacuaaccaugaugauucuagaagaacucgguucacugucuga

SEQ ID NO: 6 - protein, 201 aa, Brassica rapa
MATEDVNEALAAAEVPATETTEKQPADKLERKWSFWFDNQSKPKQGAAWGASLRKAYTFDTVQDFWGVCLSSPFTYCRSVKLDLLLQFARDYIHPQTDAECNSHVQSWCAVGRSVCWRKVDFCCYLQPQACFRQGLANFDGSCRRAIGDLWGGCCAPKAGQALLVDKDQISCSDGYWEEVEGDTCHRQDNFHPFKNSVHCL

SEQ ID NO: 7 - RNA, 615 nt, Brassica rapa
auggcgacagaggaugugaacgaagcccuugcggcggcggaaguaccggcaacagagacgacggagaagcagccugcugacaagcucgaaagaaaguggaguuucugguucgauaaccaauccaaaccaaagcaaggcgccgccuggggagccucccuucgcaaagccuauaccuucgacaccguccaagacuucugggggaucuucuuuugcaguuugcacgagacuauauucaucccuagcaaacugacgccgaaugcugaaauucacauguucaaagcugguguugagccuaagugggaagauccugagugugcuaauggcggaaaguggacuuuuguuguuaccuccaaccgcaagccugcuuuagacaaggcuuggcuugaaacuuugauggcucuugucggagagcaauuugaugaggcugaugagaucuguggggugguugcuagugugcgcccaaagcaggacaagcucuccuuguggacaaggaccaaaucuaaugaagcuguucugauggguauugggaagaaguggaaggagauacuugaugucaccgacaagauaacuuucacuaaccaugaugauucuagaagaacuagguucacugucuga

SEQ ID NO: 8 - protein, 204 aa, Brassica rapa
MATEDVNEALAAAEVPATETTEKQPADKLERKWSFWFDNQSKPKQGAAWGASLRKAYTFDTVQDFWGIFFCSLHETIFIPSKLTPNAEIHMFKAGVEPKWEDPECANGGKWTFVVTSNRKPALDKAWLETLMALVGEQFDEADEICGVVASVRPKQDKLSLWTRTKSNEAVLMGIGKKWKEILDVTDKITFTNHDDSRRTRFTV

SEQ ID NO: 9 - RNA, 597 nt, Brassica rapa
auggcgacagaggaugugaacgaagcccuugcggcggcggaaguaccggcaacagagacgacggagaagcagccugcugacaagcucgaaagaaaguggaguuucugguucgauaaccaauccaaaccaaagcaaggcgccgccuggggagccucccuucgcaaagccuauaccuucgacaccguccaagacuucuguuugcacgagacuauauucaucccuagcaaacugacgccgaaugcugaaauucacauguucaaagcugguguugagccuaagugggaagauccugagugugcuaauggcggaaaguggacuuuuguuguuaccuccaaccgcaagccugcuuuagacaaggcuuggcuugaaacuuugauggcucuugucggagagcaauuugaugaggcugaugagaucuguggggugguugcuagugugcgcccaaagcaggacaagcucuccuuguggacaaggaccaaaucuaaugaagcuguucugauggguauugggaagaaguggaaggagauacuugaugucaccgacaagauaacuuucacuaaccaugaugauucuagaagaacucgguucacugucuga

SEQ ID NO: 10 - protein, 198 aa, Brassica rapa
MATEDVNEALAAAEVPATETTEKQPADKLERKWSFWFDNQSKPKQGAAWGASLRKAYTFDTVQDFCLHETIFIPSKLTPNAEIHMFKAGVEPKWEDPECANGGKWTFVVTSNRKPALDKAWLETLMALVGEQFDEADEICGVVASVRPKQDKLSLWTRTKSNEAVLMGIGKKWKEILDVTDKITFTNHDDSRRTRFTV

SEQ ID NO: 11 - DNA, 22 bp, Artificial Sequence
  PCR primer
atggcgacagaggatgtgaacg

SEQ ID NO: 12 - DNA, 24 bp, Artificial Sequence
  PCR Primer
tctccttccacttcttcccaatac

SEQ ID NO: 13 - DNA, 30 bp, Artificial Sequence
  RT-PCT Primer
aaaaagcaggctcgatggcgacagaggatg

SEQ ID NO: 14 - DNA, 35 bp, Artificial Sequence
  RT-PCT Primer
agaaagctgggttcagacagtgaacctagttcttc

SEQ ID NO: 15 - DNA, 35 bp, Artificial Sequence
  RT-PCR Primer
agaaagctgggttcagacagtgaaccgagttcttc

SEQ ID NO: 16 - DNA, 36 bp, Artificial Sequence
  PCR Primer
aaaaagcaggcttttggtctgcagttatgttattag

SEQ ID NO: 17 - DNA, 30 bp, Artificial Sequence
  PCR Primer
agaaagctgggtaaaaaggcttgcgagtca

SEQ ID NO: 18 - DNA, 20 bp, Artificial Sequence
  PCR Primer
caatggcggtagaagacact

SEQ ID NO: 19 - DNA, 20 bp, Artificial Sequence
  PCR Primer
agttgagtttttgttcttac

SEQ ID NO: 20 - DNA, 36 bp, Artificial Sequence
  PCR Primer
aaaaagcaggcttaggacaaatgatatggggagagt

SEQ ID NO: 21 - DNA, 30 bp, Artificial Sequence
  PCR Primer
agaaagctgggtagcttggcgaccttttga

SEQ ID NO: 22 - DNA, 21 bp, Artificial Sequence
  PCR Primer
tgaaaggggcgaaaaacacat

SEQ ID NO: 23 - DNA, 24 bp, Artificial Sequence
  PCR Primer
gcaaaccgacaaaataaggaagaa

SEQ ID NO: 24 - DNA, 34 bp, Artificial Sequence
  PCR Primer
aaaaagcaggcttttttaagaatggagggagtat

SEQ ID NO: 25 - DNA, 29 bp, Artificial Sequence
  PCR Primer
agaaagctgggtgaagcgcgggtcaaaat

SEQ ID NO: 26 - DNA, 36 bp, Artificial Sequence
  PCR Primer
aaaaagcaggcttttggtctgcaattatcttattag

SEQ ID NO: 27 - DNA, 30 bp, Artificial Sequence; identical to SEQ ID NO: 17
  PCR Primer

SEQ ID NO: 28 - DNA, 36 bp, Artificial Sequence; identical to SEQ ID NO: 20
  PCR Primer

SEQ ID NO: 29 - DNA, 30 bp, Artificial Sequence; identical to SEQ ID NO: 21
  PCR Primer

SEQ ID NO: 30 - DNA, 21 bp, Artificial Sequence
  PCR Primer
tgaaaggggcgaaaaacacat

SEQ ID NO: 31 - DNA, 24 bp, Artificial Sequence
  PCR Primer
gcaaaccgacaaaataaggaagaa

SEQ ID NO: 32 - DNA, 32 bp, Artificial Sequence
  PCR Primer
aaaaagcaggctcgaagaagtccgcataaagc

SEQ ID NO: 33 - DNA, 32 bp, Artificial Sequence
  PCR Primer
agaaagctgggtacccgtccgtggattaaata

SEQ ID NO: 34 - DNA, 1157 bp, Brassica rapa
atggcggtagaagacacactcaagcctaatgtcgctacggaagaatcgaatcccaattctgcagatcacccgatcgatcgataccatgaggaaggcgacgatgccgaggaaggagcgaccgtagacgaatcgagcaaatccgccgtccctgaatcgcatccgttggagcattcgtggactctctggttcgataacccttccgtcaaatcaaagcagacgacttggggaagctccttacgatccgtcttcaccttctccaccgtcgaggagttctggaggttggtagctttacaacaatctttttccttcttacagtaattccacaatctgggttttgtttagattttgatttctcacaggaaagttatcttctttgttgttgctgttagaatcttgtttgatgtttgaacaaacagttacttgttggatgctagtgtattggctttgacattttacttttgatttgtagtttgtacaataacattcggcacccgagcaagttagctaacggagctgacttgtactgtttcaaacacaatattgaacctaagtgggaggatcctatctgtgccaacggaggcaagtggactatgaacttctctagggagaagtctgataagccctttctttacaccgtatgtaacttgacattcatatagttcttgtttcacaccatccagtctccagtctaatcgggttgttgttgttgttgttgtcacttgtagttgcttgctttgattggagaacagtttgaccatggagatgaaatctgtggagttgttgttaacgttagagctaagcaagagaggatatctatttggactaaaaactcttccaacgaagcggctcaggtacaagacaaaaaaaacccacatcaaactgtgtctctctctcggtctgaagaaaagacgtggaaattttattttatttaatgttacaggtgagcattgggagacagtggaaggagtttcttgattacaacagcagcattggtttcatcatccatgtaaagagcgtttctgttgttgctaatttctgttttttttttctttctatggatcgctcactacttgttgtatgtgtgtattggtttggtttctcttcaggaggatgcgaagaagctggacagaggcgcaaagagcgcttacactgcctga

SEQ ID NO: 35 - RNA, 687 nt, Brassica rapa
auggcgguagaagacacacucaagccuaaugucgcuacggaagaaucgaaucccaauucugcagaucacccgaucgaucgauaccaugaggaaggcgacgaugccgaggaaggagcgaccguagacgaaucgagcaaauccgccgucccugaaucgcauccguuggagcauucguggacucucugguucgauaacccuuccgucaaaucaaagcagacgacuuggggaagcuccuuacgauccgucuucaccuucuccaccgucgaggaguucuggaguuuguacaauaacauucggcacccgagcaaguuagcuaacggagcugacuuguacuguuucaaacacaauauugaaccuaagugggaggauccuaucugugccaacggaggcaaguggacuaugaacuucucuagggagaagucugauaagcccuuucuuuacaccuugcuugcuuugauuggagaacaguuugaccauggagaugaaaucuguggaguuguuguuaacguuagagcuaagcaagagaggauaucuauuuggacuaaaaacucuuccaacgaagcggcucaggugagcauugggagacaguggaaggaguuucuugauuacaacagcagcauugguuucaucauccaugaggaugcgaagaagcuggacagaggcgcaaagagcgcuuacacugccuga

SEQ ID NO: 36 - protein, 228 aa, Brassica rapa
MAVEDTLKPNVATEESNPNSADHPIDRYHEEGDDAEEGATVDESSKSAVPESHPLEHSWTLWFDNPSVKSKQTTWGSSLRSVFTFSTVEEFWSLYNNIRHPSKLANGADLYCFKHNIEPKWEDPICANGGKWTMNFSREKSDKPFLYTLLALIGEQFDHGDEICGVVVNVRAKQERISIWTKNSSNEAAQVSIGRQWKEFLDYNSSIGFIIHEDAKKLDRGAKSAYTA

SEQ ID NO: 37 - DNA, 1189 bp, Brassica rapa
atggcggtagaagacactctcaagcctaacgtccctacggaagaatcgaatcccaattctgtagatcacccgatcgatcgataccatgaggaaggcgacgatgccgaggaaggagcgatcgtagacgaatcgagcaaatccgccgtccctgaatcgcatccgttggagcattcgtggactctctggttcgataacccttccgtcaaatcaaagcagacgacttggggaagctccttacgatccgtcttcaccttctccaccgtcgaggagttctggaggttggtagctttacaacaatctttttccttcttaatgtaattccacaatctgggttttgtttagatttcgatttctcacaggaaagttatcttctttatgggtgggtttaaatctcatgaagtcactgttcttctctgtctatgaagaattgcctgtttggtgtttgaacaaacagttacttgttggatgctattttattggcttcttattatatgtgacattgcagtttgtacaataacattcggcatccgagcaagttagctaacggagctgacttgtactatttcaaacacaatattgaacctaagtgggaggatcctatctgtgccaacggaggcaagtggactatgaacttctctagggagaagtctgataagccctttctttacaccgtatgtaacttgacattcatatagttcttgtttcacaccatccagtctccagtctaatcgggttgttgttgttgttgtcacttatagttgcttgctttgattggagaacagtttgaccatggagatgaaatctgtggagttgttgttaacgttagagctaagcaagaaaggatatctatttggactaaaaactcttccaacgaagctgctcaggtacaagacaaaaaaagaacccccatcgaactgtatctctctctcggtctgaagaaaagacgtggaaattttatattgtttaatgttacaggtgagcattgggagacagtggaaggagtttcttgattacaacagcagcattggtttcatcatccatgtaatagtatttctgttgttgctaatttctttctttttttcttctatggatcgctcactacttgttgtatgtgtgtattggtttggtttctcttcaggaggatgcgaagaagctggacagaggcgcaaagagcgcttacactgcctga

SEQ ID NO: 38 - RNA, 687 nt, Brassica rapa
auggcgguagaagacacucucaagccuaacgucccuacggaagaaucgaaucccaauucuguagaucacccgaucgaucgauaccaugaggaaggcgacgaugccgaggaaggagcgaucguagacgaaucgagcaaauccgccgucccugaaucgcauccguuggagcauucguggacucucugguucgauaacccuuccgucaaaucaaagcagacgacuuggggaagcuccuuacgauccgucuucaccuucuccaccgucgaggaguucuggaguuuguacaauaacauucggcauccgagcaaguuagcuaacggagcugacuuguacuauuucaaacacaauauugaaccuaagugggaggauccuaucugugccaacggaggcaaguggacuaugaacuucucuagggagaagucugauaagcccuuucuuuacacguugcuugcuuugauuggagaacaguuugaccauggagaugaaaucuguggaguuguuguuaacguuagagcuaagcaagaaaggauaucuauuuggacuaaaaacucuuccaacgaagcugcucaggugagcauugggagacaguggaaggaguuucuugauuacaacagcagcauugguuucaucauccaugaggaugcgaagaagcuggacagaggcgcaaagagcgcuuacacugccuga

SEQ ID NO: 39 - protein, 228 aa, Brassica rapa
MAVEDTLKPNVPTEESNPNSVDHPIDRYHEEGDDAEEGAIVDESSKSAVPESHPLEHSWTLWFDNPSVKSKQTTWGSSLRSVFTFSTVEEFWSLYNNIRHPSKLANGADLYYFKHNIEPKWEDPICANGGKWTMNFSREKSDKPFLYTLLALIGEQFDHGDEICGVVVNVRAKQERISIWTKNSSNEAAQVSIGRQWKEFLDYNSSIGFIIHEDAKKLDRGAKSAYTA

SEQ ID NO: 40 - DNA, 910 bp, Brassica rapa
atggcggtagaagacactttcaagcctgttgttgctatcaaggaagcgaaacctaattatgtagagcatctgattggaccaggcgacgatgcggaggaaggagagatcgtagacggagatgttgacaaatctggaaatccacagttcctgaatcgcattcgttggagcatttgtggactttccacagttcctctttttattcgttgactttctaacgaaaagacgacttggggaagctccttagatccgcgttcacgttctccacggtcgaggagttctggaggttggtgctttaaaacaatcttttcgttcttccaataattctacaatctgggttttggtttggatttagatttctcgaggaaagttatgttctttgttgatgggttagatcacatgaagtcatcgttcttatctgtttctgaagaattgtttgtttgatgtttgaatttgtagctacaagcttatatgttaagtttttaaaaagatagcgaagatattatattcgatgtaaatcaatgttttacaccttagtatttttgttggtaacagaagatgaacaaagagttatttggttagtgttggatgctattgtattgctgtgcactcgtgtgtgtatatgctttcttgtattctcctttcttgagaacctttctctcaatgggaataatgaacttgtagtttgttctattgggagacaatagaaggagttccttgattacaacagctgcattggtttcatcatccatgtgggaagagtgcttgtcttgatgctaattcaaaaggcttttcttttgcatttctcagtgtttatttttttgtctgtattggcttgttttcccttcaggaggatgcgacgaagatgaacaagtacaaccatactgttatcgatctacaatttgagttttaa

SEQ ID NO: 41 - RNA, 404 nt, Brassica rapa
auggcgguagaagacacuuucaagccuguuguugcuaucaaggaagcgaaaccuaauuauguagagcaucugauuggaccaggcgacgaugcggaggaaggagagaucguagacggagauguugacaaaucuggaaauccacaguuccugaaucgcauucguuggagcauuuguggacuuuccacaguuccucuuuuuauucguugacuuucuaacgaaaagacgacuuggggaagcuccuuagauccgcguucacguucuccacggucgaggaguucuggagugggagacaauagaaggaguuccuugauuacaacagcugcauugguuucaucauccaugaggaugcgacgaagaugaacaaguacaaccauacuguuaucgaucuacaauuugaguuuuaa

SEQ ID NO: 42 - protein, 132 aa, Brassica rapa
MAVEDTFKPVVAIKEAKPNYVEHLIGPGDDAEEGEIVDGDVDKSGNPQFLNRIRWSICGLSTVPLFIRLSNEKTTWGSSLDPRSRSPRSRSSGVGDNRRSSLITTAALVSSSMRMRRRTSTTILLSIYNLSF

SEQ ID NO: 43 - DNA, 1567 bp, Brassica rapa
atggcggtagaagacacttccaagcctgttgtcgttgcggaagaagcgaaccctaaccccacagaccatccgattgatcgataccatgaagaaggcgacgatgctgaggaaggagagatcgccggcggcgaaggagacggagacgaatcgagcaaatccgccgttccgcagtcgcatccgttggagcattcgtggactttctggttcgataacccttctgttaaattaaagcaggcgacttggggaagctccttgcgatccgtgttcactttctccaccgtcgaggagttctggaggttagggctttttacaaaatcaataatttattcttacaattattatttcgacatgggttttagtttggttttgtctagattatgttttctcgaagaaagttatgttctttcttcgtgggttaagtgaatcacttgttcttgtttgtttctgaaatattgctttgcttgtttgtttggtgtttgaattatggaaaaggaatcttttgttctttcaatgactatgcggcatgggttttggtttagttttgtttagattgttatatctcaaggaaagttatgttctttgttggtgggttagattccgtgaagtcacttgctcttgtatgtttctgaagaatcacttaattggtgtttgagtttgtagctactgcttatatgttaaggtcatatttgttcgcttgttatcttcacaagagctaaaacattgaaccagggaatcatcggtcttattcggttaatgttggatgctattgtgttgttgcgtgtgtgtatatatactttcttgtgttcttctttttgatttgtgagtctctctcaagtctcaatgggatttaaggacttgtctttggctctattgacttcatcttactttggttgcagtctgttcaataacatgaggggtccgagcaagttagctggcggagctgacttctactgtttcaagcacaatatcgaacctaagtgggaggatcctatctgtgctaatggaggcaaatggactatgaacttcccgaaggagaagtctgataagccctggctttacaccgtatggttttgattcttcttacttgaacacatgattcttgtttcaccatccattcgagtctgattgggtttttgttttctcgatgtagttgcttgcgttgattggagaacagtttgaccatggagatgagatatgcggagctgttgtcaacgttagaggaaagcaagagaggatttccatttggaccaaaaatgcttccaacgaagctgctcaggtaaaagatcatttattgacaaataaatgttaaattgtctctcttccggctaaaagacctgaaatttcttgtttcctttgatgttgcaggtgagcattgggaaacaatggaaggagtttattgattacaacaacagcattggtttcatcatccatgtaagaagagagcttttctcttgaatgcttattcataagtttttttttaatatctcactgtctgtattgttttttttttcttcaggaggatgccaagaagctggacaggggcgcgaagagcgcttacaccgcttga

SEQ ID NO: 44 - RNA, 705 nt, Brassica rapa
auggcgguagaagacacuuccaagccuguugucguugcggaagaagcgaacccuaaccccacagaccauccgauugaucgauaccaugaagaaggcgacgaugcugaggaaggagagaucgccggcggcgaaggagacggagacgaaucgagcaaauccgccguuccgcagucgcauccguuggagcauucguggacuuucugguucgauaacccuucuguuaaauuaaagcaggcgacuuggggaagcuccuugcgauccguguucacuuucuccaccgucgaggaguucuggagucuguucaauaacaugagggguccgagcaaguuagcuggcggagcugacuucuacuguuucaagcacaauaucgaaccuaagugggaggauccuaucugugcuaauggaggcaaauggacuaugaacuucccgaaggagaagucugauaagcccuggcuuuacaccuugcuugcguugauuggagaacaguuugaccauggagaugagauaugcggagcuguugucaacguuagaggaaagcaagagaggauuuccauuuggaccaaaaaugcuuccaacgaagcugcucaggugagcauugggaaacaauggaaggaguuuauugauuacaacaacagcauugguuucaucauccaugaggaugccaagaagcuggacaggggcgcgaagagcgcuuacaccgcuuga

SEQ ID NO: 45 - protein, 234 aa, Brassica rapa
MAVEDTSKPVVVAEEANPNPTDHPIDRYHEEGDDAEEGEIAGGEGDGDESSKSAVPQSHPLEHSWTFWFDNPSVKLKQATWGSSLRSVFTFSTVEEFWSLFNNMRGPSKLAGGADFYCFKHNIEPKWEDPICANGGKWTMNFPKEKSDKPWLYTLLALIGEQFDHGDEICGAVVNVRGKQERISIWTKNASNEAAQVSIGKQWKEFIDYNNSIGFIIHEDAKKLDRGAKSAYTA

SEQ ID NO: 46 - DNA, 1568 bp, Brassica rapa
atggcggtagaagacacttccaagcctgttgtcgttgcggaagaagcgaaccctaaccccacagaccatccgattgatcgataccatgaagaaggcgacgatgttgaggaaggagagatcgccggcggcgaaacagacggagacgaatcgagcaaatccgccgttccgcagtcgcatccgttggagcattcgtggaccttctggttcgataacccttctgttaaattaaagcaggcgacttggggaagctccttgcgatccgtgttcactttctccaccgtcgaggagttctggaggttagggctttttacaaaatcaataatttattcttgcaatgattatttcgacatgggttttagtttggttttgtctagattatgttttctcgaggaaagttatgttctttcttcgtgggttaagtcaagtcacttgttcttgtctgtttctgaagtatgacttgtttggtgtttgaattatggaggtcaggccttacaaaacaatcttttgttcttcttctgattatttcgacatgggttttagtttggttttgtctagattatgttttctcgaggaaagttatgttctttcttgttgggttaagtgaagtcacttgctcttgtctgtttctgaaatattacttgtttggtgtttgaaattgtagctactgcttatatgttaaggtcatatttgttcacttctaatcttcacaagagctaaaacattgaactagggaatcattggtcttatttggttaatgttggatgctattgtgttgttgcgtgtgtgtatatatactttcttgtgttcttctttttgatttgtgagtctctctcaagtctcaatgggatttaaggacttgtctttggctctattgacttcatcttactttggttgcagtctgttcaataacatgaagggtccgagcaagttagctggcggagctgacttctactgtttcaagcacaatatcgaacctaagtgggaggatcctatctgtgctaatggaggcaaatggactatgaacttcccgaaggagaagtctgataagccctggctttacactgtatggttttgattcttcttacttgaacacatgattcttgtttcaccatccattcgagtctgattgggtttttgttttttccatgtagttgcttgcgttgattggagaacagtttgaccacggagatgagatatgcggagctgttgtcaacgttagaggaaagcaagagaggatttccatttggaccaaaaatgcttccaacgaagctgctcaggtaaaagatcatttattgacaaataaatgttaaattgtctctcttccggctaaaagacctgaaatttcttgtttcctttgatgttgcaggtgagcattgggaaacaatggaaggagtttattgattacaacaacagcattggtttcatcatccatgtaagaagagagcttttctcttgaatgcttattcataagtttttttttaatatctcactgtctgttttgttttttttttcttcaggaggatgccaagaagctggacaggggcgcgaagagcgcttacaccgcttga

SEQ ID NO: 47 - RNA, 705 nt, Brassica rapa
auggcgguagaagacacuuccaagccuguugucguugcggaagaagcgaacccuaaccccacagaccauccgauugaucgauaccaugaagaaggcgacgauguugaggaaggagagaucgccggcggcgaaacagacggagacgaaucgagcaaauccgccguuccgcagucgcauccguuggagcauucguggaccuucugguucgauaacccuucuguuaaauuaaagcaggcgacuuggggaagcuccuugcgauccguguucacuuucuccaccgucgaggaguucuggagucuguucaauaacaugaaggguccgagcaaguuagcuggcggagcugacuucuacuguuucaagcacaauaucgaaccuaagugggaggauccuaucugugcuaauggaggcaaauggacuaugaacuucccgaaggagaagucugauaagcccuggcuuuacacuuugcuugcguugauuggagaacaguuugaccacggagaugagauaugcggagcuguugucaacguuagaggaaagcaagagaggauuuccauuuggaccaaaaaugcuuccaacgaagcugcucaggugagcauugggaaacaauggaaggaguuuauugauuacaacaacagcauugguuucaucauccaugaggaugccaagaagcuggacaggggcgcgaagagcgcuuacaccgcuuga

SEQ ID NO: 48 - protein, 234 aa, Brassica rapa
MAVEDTSKPVVVAEEANPNPTDHPIDRYHEEGDDVEEGEIAGGETDGDESSKSAVPQSHPLEHSWTFWFDNPSVKLKQATWGSSLRSVFTFSTVEEFWSLFNNMKGPSKLAGGADFYCFKHNIEPKWEDPICANGGKWTMNFPKEKSDKPWLYTLLALIGEQFDHGDEICGAVVNVRGKQERISIWTKNASNEAAQVSIGKQWKEFIDYNNSIGFIIHEDAKKLDRGAKSAYTA

SEQ ID NO: 49 - DNA, 1283 bp, Brassica rapa
atggcgacggaggatgtgaacgaagcccttgcggcggcggaagtaccgatagagtcgacaacggagaagcagcctcataagctggaaagaaaatggtgtttctggttcgataaccaatctaagccaaagcaaggcgccgcctggggagcttcccttcgtaaagcctctaccttcgacactgtcgaagatttctgggggtgtgtcgtgtcttcttctcctcctcatttttagatttcttcgattaacttcttctggcatgcgtttttgcagtttgcacgagactatattcattcccagcaaattgacacccaatgctgatatccacttgttcaaagctggcgttgagcccaagtgggaagatcctgagtgtgctcacggcggaaagtggacttttgttgtcaccaacaacaggaagcaagctttagacaaggcttggcttgaaactgtaataccgtcttcccttttactgtttttgtctttagacaattgtggcttatgtcctaatgtctgtttcttctctctctctctcgtaattgggcggcagttgatggctttgattggagagcaattcgatgaggcagatgagatttgtggtgttgttgctagtgtgcgcctaaagcaagacaagctctccttgtggacacggactaaatcaaatgaagctgtcctggttagattacgaatcatgttttcttctagttgtcttttttttttttttttttcattttcttgctttttggtggtgtgcgatgagatgcccaagtactattcactagcttcctttgttgaacgtgttgattgctttctacagtaaaatagcataagctgtttaatatatcaataacgctactctaaattatcaacgaaagatgtagagaggttttttataatgagttaaattagtttttatactgaaggtttataggttcgtttaactattcatatttctgtgatacctgcttttatagtttacgctctataaacatagcatttgacagctctttagaacatggcagtatctagatgctaaaagactagtttctgaatctgtctgcttaaattactgctttgttgtttgttatggtaaattcagatgggtattggaaagaagtggaaggcgctacttgacgtcaccgacaagataactttcactaaccatgtaattaacgttctcctatagaagctaatattacttttgttcatgtttatcctttcacgtgcttactaaaatctggtctacttacttgcaggatgattctagaagaagtcggttcactgtctga

SEQ ID NO: 50 - RNA, 597 nt, Brassica rapa
auggcgacggaggaugugaacgaagcccuugcggcggcggaaguaccgauagagucgacaacggagaagcagccucauaagcuggaaagaaaaugguguuucugguucgauaaccaaucuaagccaaagcaaggcgccgccuggggagcuucccuucguaaagccucuaccuucgacacugucgaagauuucugggguuugcacgagacuauauucauucccagcaaauugacacccaaugcugauauccacuuguucaaagcuggcguugagcccaagugggaagauccugagugugcucacggcggaaaguggacuuuuguugucaccaacaacaggaagcaagcuuuagacaaggcuuggcuugaaacuuugauggcuuugauuggagagcaauucgaugaggcagaugagauuugugguguuguugcuagugugcgccuaaagcaagacaagcucuccuuguggacacggacuaaaucaaaugaagcuguccugauggguauuggaaagaaguggaaggcgcuacuugacgucaccgacaagauaacuuucacuaaccaugaugauucuagaagaagucgguucacugucuga

SEQ ID NO: 51 - protein, 198 aa, Brassica rapa
MATEDVNEALAAAEVPIESTTEKQPHKLERKWCFWFDNQSKPKQGAAWGASLRKASTFDTVEDFWGLHETIFIPSKLTPNADIHLFKAGVEPKWEDPECAHGGKWTFVVTNNRKQALDKAWLETLMALIGEQFDEADEICGVVASVRLKQDKLSLWTRTKSNEAVLMGIGKKWKALLDVTDKITFTNHDDSRRSRFTV

SEQ ID NO: 52 - DNA, 1283 bp, Brassica rapa; identical to SEQ ID NO: 49

SEQ ID NO: 53 - RNA, 597 nt, Brassica rapa; identical to SEQ ID NO: 50

SEQ ID NO: 54 - protein, 198 aa, Brassica rapa; identical to SEQ ID NO: 51

SEQ ID NO: 55 - DNA, 1148 bp, Brassica rapa
atggcgacagaggatgtgaacgaagcccttgcggcggcggaggtaacggcgatagaatcgacggagaagcagcagcctcctcacaagctcgaaagaaagtggagtctctggttcgataaccaatcgaaacccaagcaaggcgccgcctggggagtttccctccgtaaagcatgtaccttcgataccgtcgaagacttctgggggtttgtctttttcttcttcgatctaagattttctgtgaagttatactaataagggtgtgtgtattgttgcagtttgcacgagactatcttcgttcccagcagattgacacccaacgctgacattcacatgttcaaagctggtgttgagcccaagtgggaagatcctgagtgtgctaacggcggaaagtggacttatgttgttaccaacaacaggaagcaagctttagacaaggcttggcttgaaactgtactcttcttcttcttctaaccctttttactcttctgttttctgacttaataattttatctcttgtgtttggcagttgatggctttagttggagagcagtttgatgaggcagatgagatctgtggtgtggttgctagtgtccgccaaaagcaagacaagctctccttgtggactaggactaaatctaatgaagctgttctggtatcatgcttctcttctcccttatatatgtttgtttgacagttttttaaaccaccttttgatactttgctgacagtataatcataagctatatttgccaaaggatatatatatatcagtttagaacatgttagtatgtcaaagatggtttatgaatctatctatcggatgaaattgctgcttgttgtttgtttattgttattatgttttatattggtttatgatcctatctgatgagatttctactctgctgtatatttagattgatttatgaatttatctgatgaaactactacactttgttgtaaacctagatgggtattgggaagaagtggaaggagatacttgatgtcactgacaagatatctttcactaaccatgtaattactacttccccacgtaaaaagctaataaatcatccttttgttagttcctttttaaactgtggtctaaatatatgcaggatgatgcaagaagaagtcgatttagtgtctaa

SEQ ID NO: 56 - RNA, 603 nt, Brassica rapa
auggcgacagaggaugugaacgaagcccuugcggcggcggagguaacggcgauagaaucgacggagaagcagcagccuccucacaagcucgaaagaaaguggagucucugguucgauaaccaaucgaaacccaagcaaggcgccgccuggggaguuucccuccguaaagcauguaccuucgauaccgucgaagacuucugggguuugcacgagacuaucuucguucccagcagauugacacccaacgcugacauucacauguucaaagcugguguugagcccaagugggaagauccugagugugcuaacggcggaaaguggacuuauguuguuaccaacaacaggaagcaagcuuuagacaaggcuuggcuugaaacuuugauggcuuuaguuggagagcaguuugaugaggcagaugagaucuguggugugguugcuaguguccgccaaaagcaagacaagcucuccuuguggacuaggacuaaaucuaaugaagcuguucugauggguauugggaagaaguggaaggagauacuugaugucacugacaagauaucuuucacuaaccaugaugaugcaagaagaagucgauuuagugucuaa

SEQ ID NO: 57 - protein, 200 aa, Brassica rapa
MATEDVNEALAAAEVTAIESTEKQQPPHKLERKWSLWFDNQSKPKQGAAWGVSLRKACTFDTVEDFWGLHETIFVPSRLTPNADIHMFKAGVEPKWEDPECANGGKWTYVVTNNRKQALDKAWLETLMALVGEQFDEADEICGVVASVRQKQDKLSLWTRTKSNEAVLMGIGKKWKEILDVTDKISFTNHDDARRSRFSV

SEQ ID NO: 58 - DNA, 1128 bp, Brassica rapa
atggcgacagaggatgtgaacgaagcccttgcggcggcggaggtaacggcgatagaatcgacggagaagcagcagcctcctcacaagctcgaaagaaagtggagtttctggttcgataaccaatcgaaacccaagcaaggcgccgcctggggagcttccctccgtaaagcatgtaccttcgataccgtcgaagacttctgggggtttgtctttttcttcttcgatctaagattttctgtgaagttatactaataggggtgtgtgtattgttgcagtttgcacgagactatcttcgttcccagcagattgatacccaacgctgacattcacatgttcaaagctggtgttgagcccaagtgggaagatcctgagtgtgctaacggcggaaagtggacttatgttgttaccaacaacaggaagcaagctttagacaaggcttggcttgaaactgtactcttcttcttcttctaaccctttttactcttctgttttctgacttaataattttatctcttgtgtttggcagttgatggctttagttggagagcagtttgatgaggcagatgagatctgtggtgtggttgctagtgtccgcccaaagcaagacaagctctccttgtggactaggactaaatctaatgaagctgttctggtatcatgcttctcttctcccttatatatgtttgtttgacagttttttaaaccaccttttgatactttgctgacagtataatcataagctatatttgccaaaggatatgttagtatgtcaaagatggtttatgaatctatatatctgatgaaattgttgtttgttgtttgtttattgttattatgttttatattggtttatgatcctatctgatgagatttctactctgctatatatttagattggtttatgaatttatctgacgaaactaatacactttgtttgtaaacctagatgggtattgggaagaagtggaaggagatacttgatgtcaccgacaagatatctttcactaaccatgtaattactacttccccacgtaaaaagctaatcaatcatccttttgttagtgcctttttaaactgtggtctatgtatatgcaggatgatgcaagaagaagtcgatttagtgtctga

SEQ ID NO: 59 - RNA, 603 nt, Brassica rapa
auggcgacagaggaugugaacgaagcccuugcggcggcggagguaacggcgauagaaucgacggagaagcagcagccuccucacaagcucgaaagaaaguggaguuucugguucgauaaccaaucgaaacccaagcaaggcgccgccuggggagcuucccuccguaaagcauguaccuucgauaccgucgaagacuucugggguuugcacgagacuaucuucguucccagcagauugauacccaacgcugacauucacauguucaaagcugguguugagcccaagugggaagauccugagugugcuaacggcggaaaguggacuuauguuguuaccaacaacaggaagcaagcuuuagacaaggcuuggcuugaaacuuugauggcuuuaguuggagagcaguuugaugaggcagaugagaucuguggugugguugcuaguguccgcccaaagcaagacaagcucuccuuguggacuaggacuaaaucuaaugaagcuguucugauggguauugggaagaaguggaaggagauacuugaugucaccgacaagauaucuuucacuaaccaugaugaugcaagaagaagucgauuuagugucuga

SEQ ID NO: 60 - protein, 200 aa, Brassica rapa
MATEDVNEALAAAEVTAIESTEKQQPPHKLERKWSFWFDNQSKPKQGAAWGASLRKACTFDTVEDFWGLHETIFVPSRLIPNADIHMFKAGVEPKWEDPECANGGKWTYVVTNNRKQALDKAWLETLMALVGEQFDEADEICGVVASVRPKQDKLSLWTRTKSNEAVLMGIGKKWKEILDVTDKISFTNHDDARRSRFSV

SEQ ID NO: 61 - DNA, 24 bp, Brassica rapa
tctccttccacttcttcccaatac

SEQ ID NO: 62 - DNA, 24 bp, Brassica rapa
tagacaaggcttggcttgaaactg